European Patent Application EP 4 273 209 A1, published November 8, 2023. Title: MACHINE-CLEANING COMPOSITIONS CONTAINING ENZYMES. Applicant: The Procter & Gamble Company. The sequence listing filed with the application follows.

SEQUENCE LISTING (67 sequences)

SEQ ID NO: 1 - protein, 288 aa, Flavobacterium sp.
MSIQFSKILLLTVLATATISNAQDKKSKSKTAKIDWSHWTVTVPEENPDKPGKPYSLGYPEILNYAEDKIASKYMYDDPKDKSVVFYAFPSGVTTANTHYSRSELRETMETGSNKVNWTFAKGGKMRGTYAIDDISKEPDGKYSRVIIAQIHGVLTDEQRDLIGQKDNNAPPILKVYWDKGKIRVKTKVLKDLNAPYKEMLLEHAWGDDEGRNFKEKIDLNTRFTLEVKVSDGRMEVILNDTESLVYDDIHMKKWGIFENYFKAGNYFQSKTPGTFAKVKIYSLQVTH

SEQ ID NO: 2 - protein, 446 aa, Zobellia galactanivorans
MKKNVFTTLRTVVNGDIMWKLIPVFFLALCLGSCSEEPVDPEEEAVLTKLSANSTAIGISSVSASTSQSPNVASNTLDGSTSTRWSGYGDGASITYDLGSSANIDYVKIAFYKGDSRKTKYEVWVGNSTSSLTKIKSKTSSGSTSDYETIDLPNSTARYIRIVGKGYVLNSGGSTVLWNSITKFQAWGSGGSSTLPISGNSPASVLGITANTWKINSFIGSPGSSATYYDDITDASGISYNTYSDDNYFYTDGEWVYFKCYRGLGGSANSQNPRVELREMDNGNLASWTGDSGTHTMEWTVQVNQLPQDTDGDGGVLCFGQIHGPSKNSDGVEVDDVVRVQFIGEENQSSGSVKLKISGYVTEEQGGSQTFSGYSLDTTYNCKLVYSGGYVELFMNGSSVFRKKMEVDDLSENYFKVGNYLQSVKGASYTGSYGLVRIKNLSVTHN

SEQ ID NO: 3 - protein, 611 aa, Saccharophagus degradans
MTFIKIMGAGALIASASLANAATFVLEKVNTGFSVDGGNGAVEARQVYLWETNTNNVNQNWVQISHGGGYYSYKKQNTNLCLDGGSGGARLQPVTLEVCDSSNYDQHWNKVKVYTGTEIYRMEKRNAPGFSIDGNGGAAARQAIYLWNSNSNNVNQQWEFIRTDEDTGDGKLAIATAFDDGSSHSSYPASKAIDGNTAWASRWAASGSPVNLTIQLEQTSRVTEVGIAWGQGGSRAYTFEIYARPGTSGSWTKVFDDVSSGSTAGIEVFDITDIDAQQIRVKTFENTAGTTWTNITEVEIYGADGGSSSSSSSSSSTSSTSSTSSTSSSSGGFNLNPNAPPSSNFNLSQWYLSVPTDTDGSGTADSIKEGELNSGYENNSYFYTGSDGGMVFKCPISGYKTSTGTSYTRTELREMLRAGNTSIATSGVNKNNWVFGSAPSSAQAAAGGVDGNMKATLAVNYVTTTGDSSQVGRVIIGQIHAEKNEPIRLYYRKLPGNSKGGIYYAHEDADGGEVWVDMIGSRSSSASNPSDGIALNEVFSYEIDVTNNMLTVKIYRDGKSTVTSQYNMVNSGYDDSDDWMYFKAGVYNQNNTGNGSDYVQATFYSLTHTHD

SEQ ID NO: 4 - protein, 307 aa, Klebsiella pneumoniae
MLKSGVMVASLCLFSVPSRAAVPAPGDKFELSGWSLSVPVDSDNDGKADQIKEKTLAAGYRNSDFFTLSDAGGMVFKAPISGAKTSKNTTYTRSELREMLRKGDTSIATQGVSRNNWVLSSAPLSEQKKAGGVDGTLEATLSVDHVTTTGVNWQVGRVIIGQIHANNDEPIRLYYRKLPHHQKGSVYFAHEPRKGFGDEQWYEMIGTLQPSHGNQTAAPTEPEAGIALGETFSYRIDATGNKLTVTLMREGRPDVVKTVDMSKSGYSEAGQYLYFKAGVYNQNKTGKPDDYVQATFYRLKATHGAQR

SEQ ID NO: 5 - protein, 248 aa, Zobellia galactanivorans
GNSPASVLGITANTWKINSFIGSPGSSATYYDDITDASGISYNTYSDDNYFYTDGEWVYFKCYRGLGGSANSQNPRVELREMDNGNLASWTGDSGTHTMEWTVQVNQLPQDTDGDGGVLCFGQIHGPSKNSDGVEVDDVVRVQFIGEENQSSGSVKLKISGYVTEEQGGSQTFSGYSLDTTYNCKLVYSGGYVELFMNGSSVFRKKMEVDDLSENYFKVGNYLQSVKGASYTGSYGLVRIKNLSVTHN

SEQ ID NO: 6 - protein, 260 aa, Flavobacterium sp.
RNGANIDLSHWTLTTPAEDPKKPGKTFDLNYPEIFDFASNDIAKKYMYEDPKDKSIVFYAYPSGTSTANSHFSRSELRETMEIGSKNVNWTFAQGGYFKGTYAIEDVSKEADGKYSRVIIAQIHGILTDSQQALIGQKDKNAAPILKIFWDQGKIRVKTKVLKNQNASLKEMLPADAWTDDKGRDFKEKIDFNTKFTLEIKVSDGRLEVIMNGTESFVYEDINIKKWGVFENYFKAGNYFQSTNPNTFAKVKIYDLQVSH

SEQ ID NO: 7 - protein, 391 aa, Flavobacterium sp.
KLVTTKLTPASVSDNGNDGNVAANTLDGNLSTRWSSDGSTGKYITYDLGSSKSISSLKIAWHQGDQRKSYFQIRVGDSTGSLTTVYDAKTTGSSGTTTALETYTLSSPVTARYVRISCFGNSLTTWNSIAETEIYSTVDDGLPDTYPTSVIGITANTWKINSFTGTPGSSAVYYDDITTASGVSYNTYNDPNYFYTDGTWTYFKCYRGLGTSSNSSNPRVELRELNNGSSASWDGSVGTHTMTWTVKVDKLPKGENGTTGVLCFGQIHGPSTNSSGVAVDDIIRVQFDGAANQSTGTVKLKISGYITEKVLGGSKSFTGYSLGTSYTFTIKYTGGKVYLYNGSTLVFSQQMDTSTEGNYFKAGNYLQSVKNVSYDGSYGLVGISSLTVSHQ

SEQ ID NO: 8 - protein, 257 aa, Pseudomonas aeruginosa
GGPSSVAFWYAERPPLAELSQFDWVVLEAAHLKPADVGYLKEQGSTPFAYLSVGEFDGDAAAIADSGLARGKSAVRNQAWNSQVMDLAAPSWRAHLLKRAAELRKQGYAGLFLDTLDSFQLQAEERREGQRRALASFLAQLHRQEPGLKLFFNRGFEVLPELPGVASAVAVESIHAGWDAAAGQYREVPQDDRDWLKGHLDALRAQGMPIVAIDYLPPERRDEARALAARLRSEGYVPFVSTPALDYLGVSDVEVQP

SEQ ID NO: 9 - protein, 906 aa, Pseudomonas seleniipraecipitans
AGLSPAGPQSVAFWYAPNPPYSELAQFDWSVLEPSHVQAKDVAFLRAQGNQPFAYLSIGEFDGDLAVVTGSASNSGASAVQNKAWGSQVMHLSSPEWRAYLLRRASELREAGYAGLFLDTLDSFQLLPAAEHETQRAALRDFLSELKRQEPGLKLFFNRGFEVLPELPGVAAAVAVESIHAGWDAQRRTYRIVPQADRDWLDGHLQPLRDKGIPLVAIEYLPPDRRNEAPALVARLVSEGFVPYVTVPNLDYLGVSTVDVQPRRIAMIFDPREGTLYQNPGHMYVGGLLEYLGYRVDYFEADQLPNRPMSGLYAGVVVWMTSGPPENALVFNQWLSARADEHVPLAFLAGLPVENDGVLRRFGLRRTFTPLTAPAEVAQQDDALIGHFEAPVVVRTRDLPSLTTLDGGPTPVLGLRDSQQRIFTPVAIGDWGGIALSPYVVEEGADQRRWIIDPFAFLQKALRLPAMPRPDTTTENGRRVATVHIDGDGFVSRAEAVGTPYSGDLVLRDFIKPYPFLTSVSVIEGEVGPRGAFPHLARELEPIARKIFAEPKVEVATHTFSHPFFWQPEVAEKREGFNPEYGYMMKIPGYDKLDFNREIAGSTAYINQNLTTPQKPVKMVFWSGDAMPDEATIKLAYDNGLTNVNGGNTALTNAYPSLTGLYPLIRPTSGGIHYYAPVINENVYTNLWTGPYYGFRGVMETFALTDKPRRLRGLHLYYHFYSGTKQASIRVMNDIYKSMAAEHPISLWMSDYVPRMHGLYQASLARRADGAWQIRGLDGLRTVRLDAAMGWPDLSRSSGVAGVRDLPQGRYVHLASGQAVLALRDTRDPRPALEEANLPLLAWTYLDDHRVKLSFAGSMPLQFSVRAQGTCRLEVAGKSYSGTRQQDLWRFSLPMERVLDAQLTCR

SEQ ID NO: 10 - protein, 904 aa, Pseudomonas sp.
AALTPPSSVTFWYAEEPPLAELAQFDWAVVEPGHMTAGDVTTLRKLGSEPFAYLSVGEFDGNKADITKAGLTAAVSPVRNDSWNSQVMDLTTQAWREYLLGRAKQLQAQGYAGLFLDTLDSFQLLPEASREAQRKALASLLRELHKRQPGLKLFFNRGFEVLPELDGVASAVAFESLYAGWDAAAKRYRPVPEADRQWLLGELAPLRAKGIPLVAIDYLPPERREEARKLAKRLRDEGYIPFISTPELNSMGISNVEVQPRRVALVYDPREGDLTVNAGHTMLGGLLEYLGYRVDYLAVDSLPEHRFSGLYAGIITWMASGPPQDGATFNRWLGKRLDEQVPVVFFAGLPTEDKVLLKRLGLNLMAPAGTQPLTISYQDKALIGAFEAPVQPRSRELTAVSLLPQGPKAALLLTGKDGQTFAPVATAKWGGLALAPYVLETNNERSRWILDPFAFLQASLQLPAQPRPDTTTENGRRIATVHIDGDGFPSRAEVRGSPYAGKQVLNDFIQPNPFLTSVSIIEGEISPRGMYPHLARELEPIARELFANPKVEVATHTFSHPFYMQPELAEKDEDFSAEYGLKMAIPGYDKIDFKREIFGSRDYINQQLTTPEKPVKMVFWPGDALPSAATIKLAYDAGLKNVNGASTMLTKARPSLTGLNPLLRPTEGGLQYYAPVINENVYTNLWKGPYYGFRDVIDTYELTDSPRRLRGIHLYYHFYSATKQASIKAMGEIYGYMREQHPMSLWMSDYLDRLHGLYQASLARTADGAWQIRGMDALRTVRLDPQMGWPDLLRSQGIAGVRDLPQGRYVHLSSDRALLVLRPDRDDRPALEEANVPLTDWRYLDDRRVSFAFAGQFDVTFSVRSASACRVEVDGQRFAGKSSAGLWTFQLPMKQVSNGQLLCN

SEQ ID NO: 11 - protein, 897 aa, Pseudomonas composti
QPASVAFWYADQLPLPELSQFEWVVVEPDHVSPGDLAYLQKQGSEVFAYLSIGEFAGDVAQAGLSEATSVVRNDAWNSQVMNLASPVWREHLFKRTSTLRQQGYTGLFLDTLDSFQLQAQDLQGSQREALKSLLSELHRREPTLKLFFNRGFEVLPELPGVASAVAVESIYAGWDAGGGYKEVSQGDRDWLLPRLDAVRKQGVPVVAIEYLPPEQREQARKLATRLTQEGFIPYVTSPALDAIGVGGVEVQPRRIALVYDAREGELEDNPGHVHLGGLLEYLGYRVDYWPADTTLPQRPLKGLYAGIVVWMTSGSPVDRDYFENWLGQRLDEQVPLAFMAGMPTENDSLLDRLGIRTRSQPVGKDAVLLSHDAALIGGFEAPLRLRTRDVPPLTVTAPERTQAALSLQSDDRVYVPVATGDWGGYALAPYVFEEGLDHRRWVLDPFAFISRAFKLPALPRPDTTTENGRRIATVHLDGDGFVSRAEVPGSPYSGIQVLEDFIKPYPLLTSVSVIEGEVGPRGMYPHLSRELEPIAREIFVNPKVEVASHTFSHPFFWQPEKATKRENFEAEYGYMMAIPGYKTLDMQREVVGARDYINQRLTTPKKPVKMIFWSGDAMPSAETIKLAYDSGLPNVNGGNTVLTKAYPSLTGLYPLIRPTTGGLHFYAPVINENVYTNLWTGPYYGFRDVQDTFALTDSPRRLRGFHLYYHFYSGTKQASIRAMRQIYQTILDGQPLSLWMSDYIKRVEGLYRASLARRSDGTWQVKGLVGMRTLRLDPSLGWPDLARSQGVAGVRDLAQGRYVHLTGADAVLALRETRDPRPALEEANIPLTGWRYLDDKRVTFSFLGEFPLSFSVRSAGACHVTAGGGRFSGTHDNGVWHFELPMKQVSDAQLVCN

SEQ ID NO: 12 - protein, 905 aa, Pseudomonas corrugata
SALPQPASVAFWYADQPPLSELAQFEWSVVEPGHMTPGDVKTLRELGSHPFAYVSVGEFDGNKAEIDKAGLRQAVSPVRNDSWNSQVMDLTAPAWREHLLGRAKALQAQGYDGLFLDTLDSFQLLPEGAREAQRVALASLLREMHKRQPTLKLFFNRGFEVLPELDGVAAAVAFESLYAGWDAAAKRYRPVPEADRQWLLGELQPLRAKGIPLVAIDYLPPERRDEARKLAKRLRDEGFIPFISTPELDSIGLSNIEVQPRRIAFVYDEREGALEDNGGHTVLGGLLEYLGYRVDYIPASSAMPGYRFSGLYAGVVTWMTSGPPQDAPAFNRWITARLDEQVPVVFFSGLPVEDKLLLKRMGLKREAPPGVQPLTITHQDKALIGAFEAPVQPRSRDLTAVSVLPNGPKPVLSLTNASGEVFTPVVTAKWGGLALAPYLLEANNERSRWIIDPFAFLQTSLQLPEQPRPDSTTENGRRVATVHIDGDGFPSRAEVRGTPYAGRHTLDDYIKPNPFLTSVSIVEGEISPRGMFPHLARELEPIAREIFANPKVEVATHTFSHPFFMQPDKALKRENFHPEYGMNMAIPGYGKIDFRREIFGSRDYINQNLTTPEKPVKMVFWPGDALPSASTLKLAYDAGLKNVNGAETMMTKANPSVTGLNPLLRPTEGGLQYYAPVINENLFTNLWKGPYYGFREVIDTFELTDSPRRLRGLHLYYHFYSSTKQASIKAMHEIYGFMREQHPLSLWMSDYIDRLHGLYQASLARTSDGAWQIRGMDALRTVRLDPGMGWPDLLRSQGIAGVRDLPQGRYVHLSSDRALLVLRPDRDDRPALEEANLPLVEWRYLDDRRVSFGFSGQFDLTFSVRSANPCRVEVDGQRFAGKAAAGLWTFQLPMKQVSHAQLVCN

SEQ ID NO: 13 - protein, 905 aa, Pseudomonas migulae
AALPQPSSVTFWYAAQPPIPELAQFDWSVVEPGHLTKDDVKTLRDLGSQPFAYVSIGEFAGSKADIEKAHLSDAISPVRNGAWDSQVMNLSAPAWREHLFGRAKTLQAEGYAGLFLDTLDSFQLQPEADREKQRLALASFLRELHQRQPTLKLFFNRGFEVLPELDGVAAAVAVESIHAGWDATAKRYRPVPEADRAWLETQLQPLRAKGIPLVAIDYLPPERRDEARKLAKRLREEGFIPYIGTPELDSMGISNIEVQPRRVALLYDLREDDLTQNDGHTLLGGLLEYLGYRVDYLPVDDTLSERRFSGLYAGVITWMTSGPPQNAAAFNTWIGKRLDEKVPVVFFAGLPIQDTSLLKRLGLNRTAPIGTQTLSITSQDKALIGAFEAPVQPRSRDLTAISLLPKGPKAALLLTAADGQTFAPVAVADWGGLALAPYILETNNERSRWILDPFAFLQASLRLPVQPRPDTTTENGRRIATVHIDGDGFPSRAEVRGTPYAGRQVYDDFIRPNPFLTSVSVIEGEISPRGMFPFLAGELEPIAREIFADPKVEVATHTFSHPFFWQPELAKKQENFSPEYGLNMAIPNYDKIDFRREIFGSRDYINQQLTTPEKPVKMVFWPGDALPSASSIKLAYDAGLKNVNGAATMLTKANPSMTGLQPLLRPTEGGLQYYAPIINENLYTNLWKGPYYGFRDVIDTFELTDSPRRMRGLHLYYHFYSSTKQASIKVMGEIYGYMKTQQPMSLWMSDYLDRLHGLYQVSLARTAEGDWQVRGLDALRTLRLDPQMGWPDLMRSQGVAGVRDLPQGRYVALSSDRALLVLRPDRDNHPALEEANLPLVDWRYVNERQVDFSFAGQVDLTFSVRLPGTCRVEVDGQHFAGKASAGLWTFQLPMKQVSHGQLFCS

SEQ ID NO: 14 - protein, 905 aa, Microbial community
AALPQPASVVFWYADQPPISELAQFDWSVVEPGHLTAGDVKTLRKLGSQPFAYLSVGEFHGGKAELEKASLTGAVSPVRNGAWDSQVMDLAAPAWREHLFGRAKALQAEGYAGLFLDTLDSFQLLPESARETQRVALAGFLRELHQRQPNLKLFFNRGFEVLPDLDGVAAAVAIESIHAGWDASAKRYRPVPEADREWLETQIQPLRAKGIPLVAIDYLPPERRDEARKLAKRLRDEGFIPYIGTPELDSMGISSIEIQPRRIALLYDPREGDLVRNAGHTLLGGLLEYLGYRVDYLPVDGSLPEHRFSGLYAGIVTWMTSGPPQDASAFNSWIGKRLDEQVPVVFFSGLPIQDPLLLKRLGLNRSAPIGTQALTISYQDKALIGAFEAPVQPRSRDLTAISLLPKGPKAALLLTAADGQTFAPVATAEWGGVALAPYILETNNERSRWILDPFAFLQASLRLPVQPRPDTTTENGRRIATVHIDGDGFPSRAEVRGTPYAGKQVLDDFIRPNPFLTSVSIVEGEISPRGMFPFLARELEPIARELFANPKVEVATHTFSHPFFMQPEVAQKRENFNPEYGLKMAIPGYDKIDFRREIFGSRDYINQQLTTPEKPVKLVFWPGDALPSAATLKLAYDAGLKNVNGAETMLTKANPSLTGLNPLLRPTEGGLQYYAPIINENLYTNLWKGPYYGFRDVIDTFELTDSPRRLRGLHLYYHFYSSTKQASIKAMNEIYGYMKDQQPMSLWMSDYLDRVHGLYQASLARTAEGDWQVRGMDALRTLRLDPQMGWPDLLRSKGVAGVRDLPQGRYVALSSDQALLVLRPDRDERPALEEANLPLVDWKYVDEKHVSFSFAGQVDLSFSVRSASSCRVEVDGQTFAAKASAGLWTFQLPMKQVSHGQLYCI

SEQ ID NO: 15 - protein, 906 aa, Pseudomonas pelagia
GPVKSGPASVAFWYAEQPPLGELAQFDWVVFEPAHLTPKDVSFVVAQGSLPFAYLSIGELNDHLAQSSPGLLDNSADQIRNPGWNSHVMDLTSAGWQEHILGQVGEFAKQGYAGVFLDTLDSFTLLPEDQRPAQRDALAALLRDMHKRYPDMKLFFNRGFEVLADVQQGVAAVAVESIYASWDAAAQVYRPVSENDRTWLAGQVQPLRARNIPIVAIDYLPVERRAEARELAARLIEEGFLPYVGTPELDTLGVSSIEVQPRRIAVMYDPREGELTRTGGFRSLGGLLEYMGYRVDYLPVEGSLPSAPMTGLYAGVIVWMTSGPPPDSSAFNRWIGRRLDEGTPLAFFQGMPIDDAAILRRLGLQRTGVQPVSGLQLVNHDAQLVGSFEAPLVVRSRGLTGIGTQSRYNKVALALVDDAGREHTPVVTGDWGGVALAPYVFEGEDDTRRWIIDPFAFLQQALQLPAQPAPDVTTENGRRIATVHIDGDGFPSRAEIPGTPYSGSAVLNQFIKPYPLLTSVSFIEGEVGPAGMYPYLSRELEPLARQILAHERVEPATHTYSHPYFWQAERDSQREGFRADYGLKMPIPGYDTIDFRREVFGSRDYVASRLAPADKPVKMIFWSGDAIPDAATIKLSYDAGMLNVNGGETRLTRADPSLTGLYPLLRPTAGGLQVYAPIINENVYTNLWQGPYYGFREVVETFELTDSPRRMRGLHLYYHFYSGTKPAAIKVMGDIYRHMLEQQPLSLWMSDYLLRAHGLHTASLARTSSGAWQIRALQGLRTVRLDPSLGWPDLMASEGIAGVLDLPQGRYVHLSADRAVLALQANRDTTPALEQANVPLTAWRYLDERRIQLSFAGEFPIAFSVRSASPCRLDVAGREVKGRGANGLWHFSLSTKQVSDAQLVCE

SEQ ID NO: 16 - protein, 266 aa, Burkholderia sp-63093
QGAADMPAGPSVALYYGANPPVEELATFDVVVVDPDAHFDPRAHAKAHPVWFAYVSVGEVNPHRAYYSAMPSAWLPGVNDAWASHVIDQTAAEWPAFFVDKVIAPLWKKGYRGFFLDTLDSYHLIAKTDAARAAQEAGLVRVIRAIKKRYPKAKLIFNRGFEVLPQIHDLAYMVAFESLYRGWDAGKQRYTEVPQADRDWLLMQAATIRDQYKLPVLSIDYCPPADDTCAAATAARITQAGFVPYVTDGGLATVGVGAAGTGNERP

SEQ ID NO: 17 - protein, 266 aa, Burkholderia sp-63093
QGPADMPAGPSVALYYGANPPVEELATFDVVVVDPDAHFDPRAHAKAHPVWFAYVSVGEVNPHRAYYSAMPSAWLPGVNDAWASHVIDQTAAEWPAFFVDKVIAPLWKKGYRGFFLDTLDSYHLIAKTDAARAAQEAGLVRVIRAIKKRYPKAKLIFNRGFEVLPQIHDLAYMVAFESLYRGWDAGKQRYTEVPQADRDWLLMQAATIRDQYKLPVLSIDYCPPADDTCAAATAARITQAGFVPYVTDGGLATVGVGAAGTGNERP

SEQ ID NO: 18 - protein, 271 aa, Paraburkholderia phenazinium
QTAADAADNAASATNASAQPSVAFFYGGQVPAAALSEFDAVVVEPDSGFDPEAQHGGHTAWFAYVSVGEVTPQRPYYAAMPKEWLVGHNAAWESKVVDQDAPGWPAFYLKQVIAPLWRKGYRGFFLDTLDSYQLIAKTDADRQRQQAGLVAVIRAIKARYPRAMLMFNRGFEILPQVHELVYAVAFESLYSGWDQTKQSYTQVPLADRDWLLGQARIIREQYRLPVISIDYCAPGDEQCARDTVQKICKDGLVPYVTDGALQTVGVGRAGR

SEQ ID NO: 19 - protein, 271 aa, Paraburkholderia phenazinium
QTAADAASNAASATNASAQPSVAFFYGGQVPAAALSEFDAVVVEPDSGFDPEAQHGGHTAWFAYVSVGEVTPQRPYYAAMPKEWLVGHNAAWESKVVDQDAPGWPAFYLKQVIAPLWRKGYRGFFLDTLDSYQLIAKTDADRQRQQAGLVAVIRAIKARYPRAMLMFNRGFEILPQVHELVYAVAFESLYSGWDQTKQSYTQVPLADRDWLLGQARIIREQYRLPVISIDYCAPGDEQCARDTVQKICKDGLVPYVTDGALQTVGVGRAGR

SEQ ID NO: 20 - protein, 882 aa, Gallaecimonas pentaromativorans
STSDSVAFFYGQHQPLAEMTFYPGVVVQPDHISAEELKWLNERGIKTYAYLSVGESDAKDAKGLKVNASWQSQIMDQTSTRWKNHLNTRAKELKARGFYGLFLDTLDSYQLLPQDQQPVQRQALLAAVQSLSGQFQHHLILNRGFELLPWLKGQAERVVAEGLLSHFNPEDNSYKGTSQADQQWLSAQLNTAKALGFAVQVIDYAPFAKRAAMAQQIAKAGFAPWVTDGHLLTWGSSELTPVPRRVIVPFDSTLKPLINTQVHQRLSTLIEYLGYLPDYIDISKEPLPPADKALFAGVVVWAESAAFYRPELVSWLEKVQGKLPELLLGEIPQSPALLAGLGLNLQSLSPKGPFSQTEMASWLKGETALSLKNLEPYSATLAEGAEALISIKAGNGEPVLQGARTDKGAVVLSPWLIDALPLEENRWLINPVALLQKGLGLPPIPAPDVTTESGRRLFTLHIDGDAFPSRARFPGQPFAGEVMEKQIIEHYQLPITVSVIQGEVGPTGMYPKQSPQLEAIARDIFTKPYVEIASHTYSHPFFWSQIAGREKLTEQDTEYGFHLNIPGYNKIDLTKEIDGSIDYINERLAPKDKKVVMMLWSGDAAPGPVALAHARKMGVLNVNGGNTVMTRDNPSLSEIWPIGRPEGDLLYQVYAPIMNENVYTDLWHGPYFGFRRVRETFDITGHPYRLKPFGLYFHFYSATNPAGLQALRDDIGYVLGRPNTPAHLSHYARMAKDFYFSALARDAKGDWLLSSKYLRTLRLPKALGYAQLDASQGLAGATEDGRYLHVVNGDARFALAASASPRKPYLVSANVLLKSWQLPGKVAFKAWQKADLILANAEGCRFVSDQGPSYGGQQKGRLTEFSLPEGDFAGHLACGTQQ

SEQ ID NO: 21 - protein, 458 aa, Thermus rehai
QVDPSHVAQAVRRTIQIGGGLEQWSGLPQYPVVLSNTFPAKPVTHGGYFSVAWDDRHLYILGVFEQKAETVKAALPEEHPEWWNDDTMEVFLKPDPKGVEVIHLAANPKGTRFKAYTFTTDYATSGRVEASRWVLEWAIPFASLKTSPPEPGAIWAMKVGREHQAAQEYPLWPMGGDYHAPTNFGYLVFVEKLEDPQALAQRVQALLGVEPPIRSRLQDIATYAVYYGKDPQEAAKLVDFDLAIVQPNLPKESLALLKANGVRVVAYLSIGEAEPERDYGQPLPKEWLLGQNPNWGSYFVDANQKGWQELVLRLAEGYLKAGFDGLFLDTLDTADLYPQVAPGLVAIVQALRERFPEAILVQNRGFRLLPKTAELVDAVMYENLSAMYNFQEKRYVAVDGDPTPVLPYAKRGLVVLALDYALPEDVDLVRRAYVRARELGFVPYVSVIRLDRVFLHNP

SEQ ID NO: 22 - protein, 277 aa, Environmental bacterial community XE
ASPALSSVGSWIYQLQGAKPDVLAASPYDMAVIDYSRDGSGGRAYSRADIAALKVKPDGGQRIVLAYLSIGEAEDYRFYWGQDWSRTPPSWLLGENPDWEGNYDIRFWDPEWQKIILGTPQSYLDRILAAGFDGVYLDRVDAYERNDREMNAPGRRAAMIAFVQDIARYGRAQNPQFLVVPQNGEELLSDAGYRQVVSGLAKEDLLYGLDGDESRNRNGEIRASLSFLNRLVAEGKPVFLAEYLSSPELIDTAHAEASELEMVLFIGDRELDNANSK

SEQ ID NO: 23 - protein, 275 aa, Tumebacillus ginsengisoli
QVKWQVNYALSTEKAVKSVSHKASSLSAVKSFMIYYGDASDSAIKKLSQYQLVIIEPRNWNGTELAQLKKSGVKVLGYLSVLEQNSNSSLLGQVQNADYLLINGKRDPRSDWDSWSMNINSGHYRDLLFADYQKEIVNKGLDGVFLDTMGDADDGIWNTSISDSQRDGAVKFVADLRNKYPSLSIMQNWGLQQLKDRTAPYIDGILWEDFTPKTVVKNAWSKSRMQELDKLHAANGLSVFTSHVGLSGAQKSKFDSLNVEHGYVGQVIKKSYDVI

SEQ ID NO: 24 - protein, 281 aa, Environmental bacterial community A
TPGMGKGILSNAKSWVYQLQHIDLPTLGTTTADLVVIDASQDGSVEGSFTPADIAALKTKPDGSQRVVLAYFSIGEAEDYRFYWDDEWYDQAPDWLHEENSDWAGNYPVKFWHPDWQAILFGSPDCYLDRIIAAGFDGVYLDRVDAFEIDDPALTRPQRAAHMIALVRSLAAYARARTPSFVVVAQNGEELLADGSYRHTVDGVGKEDLLYGLESDGKRNANGDIRVSLDYLRRLAEAGKPVFLVEYLTEPQTIAQAHADAETLGMPIFITDRDLDNAYSR

SEQ ID NO: 25 - protein, 467 aa, Myxococcus virescens
AERSEDTAGLADARTLTCASLQVASGAIGSGQSVQGLHTQTLSGTQDRWTEYVEFFPGTSATCTYALPADVGAADVIAAEVGINYRGPARSQMRWLFEAWDYAAGAWVLVGDNTFAQSWRWTATSLALTSPQRFVSGGPVKLRYRTTSTADASLLDLLVVRIQVAASDAGTPGDAGTPTDAGTPGDAGTGTDAGTPVSWEGVHSFTYQLTNYPQGKLDTIANSKFDLAIVDLSRDGYDDWFTAAEITALKAKGKQVLAYFEIGAIEEYRPEWSQVPEDLKLGPVGGWPDEQYVKYWDERWWPIVQGRLDQALAAGFTGCYLDMVVTYEEIPANAAGTNRADLARKMVALLARINQYAKARDPGFKVMPQNSPELVDDPAYLPAIDGLGMEDLYWSDDNACDEGWCEENRANAARVRAAGKLVLSTDYAVQAANVADAYTRSRAAGFVPYVSVRALDRMTVNAGWDPQ

SEQ ID NO: 26 - protein, 475 aa, Corallococcus macrosporus
RDSLDDERGAILPDAQTLTCATLQLARGSIGSGQGVQGLHTQTLSGTQDRWAEYVEFAPNSSATCTYPLPAGVSADTVVAAEIGVNFRGPTKSAMRWLFEAWDYSTGAWVVVGDNVFAQSWKWSATSLALTSPSRFFSGGPVKLRYRTESSADASLLDLLVVRVQVAATDAGTPTDAGTPTDAGTPTDAGTPTDAGTSTDAGTPVPWEGVSSFTYQLTNYPQGKLDAIAASKFDLAIVELVRDGSSGYFTAAEISALKARGKQVLAYFEIGAIEEYRPEWSQVPADLKLGPVDGWPDEQYVKYWDERWWPIVQGRIDRALAAGFTGCYLDMVVTYEEIPANAAGTNRADLARKMVALIARISQYAKARNPAFKVMPQNSPELVDDPAYLPVIDGLGMEDMYWSDDVACDASWCAENRANAARVRAAGKLVLSTDYAVQSAHVADAYTRSRAAGFVPYVTVRALDRVTVNAGWDPQ

SEQ ID NO: 27 - protein, 475 aa, Corallococcus macrosporus
RDPLDDERGAILPDAQTLTCATLQLARGSIGSGQGVQGLHTQTLSGTQDRWAEYVEFTANSSATCTYPLPSGVSADTVVAAEIGVNFRGPTKSAMRWLFEAWDYSTGAWVIVGDNAFAQSWKWSATSLALTSPARFFSGGPVKLRYRTESSADASLLDLLVVRVQVAASDAGTLTDAGTPNDAGTPTDAGTPTDAGTSTDAGTPVPWEGVSSFTYQLTNYPQGKLDAIAASKFDLAIVELVRDGSSGYFTAAEISALKTRGKQVLAYFEIGAIEEYRPEWNQVPADLKLGPVDGWPDEQYVKYWDERWWPIVQGRIDRALAAGFTGCYLDMVVTYEEIPASSAGTNRADLARKMVALIARISQYAKARNPAFKVVPQNSPELVDDPIYLPAIDGLGMEDMYWSDDVACDAGWCAENRANAARVRAAGKLVLSTDYAVQSAHVADAYTRSRAAGFVPYVTVRALDRVTVNAGWDPQ

SEQ ID NO: 28 - protein, 469 aa, Myxococcus stipitatus
RDTLDDERGAILPDAQTLTCTTLQLARGSIGSGQGVQGLHTQTLSGTQDRWAEYVEFTANSSATCTYPLPAGVSADTVVAAEIGVNFRGPTKSAMRWLFEAWDYSTGTWVVVGDNAFAQSWKWSATSLALTSPARFFSGGPVKLRYRTESSADASLLDLLVVRVQVAASDAGTSTDAGTPTDAGTPTDAGTSTDAGTPVPWEGVSSFTYQLTDYPQGKLDTIAASKFDLAIIELVRDGSSGYFTAAEISALKAGGKQVLAYFEIGAIEEYRPEWSQVPSDMKLGPVDGWPDEQYVKYWDERWWPIVQGRLDRALAAGFTGCYLDMVVTYEEIPANSAGTNRADLARKMVALIARISQYAKARNPAFKVMPQNSPELVDDPIYLPAIDGLGMEDMYWSDDVACDAGWCAENRANAARVRAAGKLVLSTDYAVQSAHVADAYTRSRAAGFIPYVTVRALDRVTVNAGWDPQ

SEQ ID NO: 29 - protein, 468 aa, Environmental bacterial community LE
DDFDTGQDAILPDARTLPCTTLQFERGALPSGQSVQGLNTQTLSGTQDRWAEYVEFAPNSSATCTYPLPTGVSADSVVAAEVGVNYRGPTKAQMRWVIEAWDYSTNSWALVGDNTFAQSWRWTATSLALPTPARFLSGGPVKLRYRTDSTADASLLDLLVVRVQVAASDAGTPTDAGTPTDAGTPTDAGTPTDAGTQVPWSNVKSFTYQLTNYPQGKLDAIAASKFDLAIVELVRDGSSGYFTAAEISALKARGKQVLAYFEIGAIEEYRPEWSQVPADLKLGPVSGWPDEQYVKYWDERWWPIVQGRIDRALAAGFNGCYLDMVVTYEEIPANSAGTNRADLARKMVALIARINTYAKARNPDFKVVPQNSPELVDDPAYLPAIDGLGMEDMYWSDDVACDEGWCEENRTNAARVRAAGKLVLSTDYATQSAHVADAYTRSRAAGFVPYVTVRALDRVTVNAGWDPQ

SEQ ID NO: 30 - protein, 464 aa, Myxococcus fulvus
ACGDKAPHDDFDTGQDAILPDARTLPCTTLQFERGALPSGQSVQGLNTQTLSGTQDRWAEYVEFAPNSSATCTHPLPTGVSADSVVAAEVGVNYRGPTKAQMRWVIEAWDYSTNSWALVGDNTFAQSWRWTATSLALPTPARFLSGGPVKLRYRTDSTADASLLDLLVVRVQVAASDAGTPTDAGTPTDAGTQVPWSNVKSFTYQLTNYPQGKLDAIAASKFDLAIVELVRDGSSGYFTAAEISALKARGKQVLAYFEIGAIEEYRPEWSQVPADLKLGPVSGWPDEQYVKYWDERWWPIVQGRIDRALAAGFNGCYLDMVVTYEEIPANSAGTNRADLARKMVALIARINTYAKARNPDFKVVPQNSPELVDDPAYLPAIDGLGMEDMYWSDDVACDEGWCEENRTNAARVRAAGKLVLSTDYATQSAHVADAYTRSRAAGFVPYVTVRALDRVTVNAGWDPQ

SEQ ID NO: 31 - protein, 467 aa, Corallococcus macrosporus
AERSGDAAVLADARTLTCASLQVASGYIGSGQTVQGLHTQTLSGTQDRWAEYVEFSPGTSATCTYALPADVGAADVVAAEVGINYRGPHKSQMRWLFEAWDYEGGAWVLVGDNTFAQSWTWTATSLALTSPQRFVSGGPVKLRYRTTSTADASLLDLLVVRIQVAASDAGTPGDAGTPGDAGTPGDAGTETDAGTPVQWEGVNSFTYQLTNYPQGKLDTIAASKFDLAIVDLARDGYDDWFTAAEIAALKAQGKQVLAYFEIGAIENYRPEWSQVPDDLKLGPVGGWPNEQYVKYWDERWWPIVQGRIDQALAAGFTGCYLDMVVTYEEIPANSAGTNRADLARKMVALIERISQYAKAHNPAFKVMPQNSPELVDDPAYLPAIDGLGMEDMYWSDDNPCDEGWCEENRTNAARVRAAGKLVLSTDYATQAAHVADAYTRSRAAGFVPYVTVRALDQMTVNAGWDPQ

SEQ ID NO: 32 - protein, 260 aa, Lysinibacillus xylanilyticus
TESTTSIQAKLADIKEYKYYLDQGNDKIGKEMANMDLVIVEPIEMQQKYIDHAQKNGTLVYGYINAMEADKWNSALYSQLNKADFYKDAHGEKMYFTEWDSYLMDMTSQHYQKLLLEEIQKQIVQKGLDGVFLDTVGNINSYLPEKEQEAQNEAMLSFIKKIKQQYNGLSVAQNWGFQTLADYTAPYIDFIMWENFSYDVVGEDDWALDRMKQLVHIRDKFGTQVMAIGFEDEEKSRALAEKYQFKFFYSPAGSHYNTWQ

SEQ ID NO: 33 - protein, 279 aa, Nonomuraea coxensis
PRVPLTEVRSFTYVLQNYPGGRLDTVARAPHQLAIVDLSRDGTTAGYFSAKEVAKVRDSGKTVLAYFEIGSIERFRTEARTLPADLRLNRWLDWPEEHFVRYWDSRWWDLVLRPRVDQALRAGFDGVYLDTPLAYEEIHLDRVPGETRASLARRMNELIVRISRYAKKVRPGFLIVPQNSPELRLQPGYVEAIDGIGMEELFFRATGRPCTTGWCAENLAHALALRKLGKAVLATDYATRPADVAAACARYRRHGIAGNVTVVDLDRVSPLCTVAKEGA

SEQ ID NO: 34 - protein, 268 aa, Lysinibacillus boronitolerans
STSIQAKLADVKDYTYYLDKGNDAIGKSMTKLDLVIVEPIEMQQKYIINAQKSGTLVYGYINAMEADKWNTALYHQLKEEDFYRDKQGERMYFAKWDSFLMDLTSTHYQDILLAEIQQQIVEKGLDGVFLDTVGNINSYLPEDEQKWQNEAILSFIQQIKKRHPDLSVAQNWGFQTLADYTAPYVDFIMWEDFSYPVVGKDEWSLDMMQQLIHIRNKFGTQVMTIGFEEESKSRALAEKHHFKFFYSPAGSYYNSWQSSLLPSDKQLF

SEQ ID NO: 35 - protein, 257 aa, Carnobacterium inhibens subsp.
EGKSNSKLENTGEYGVFLSLDGSEAIEASEGYETVIIDAQNLSEAEITEMQDRGQKVYSYLNVGSLETYRPYYEEFQYLTLRPYENWEEEYWVDVTNEDWQKFSAVTLANELLDKGIDGFWIDNVDVYWQFQTKETYIGVEKILKTLMSYGKPVLINGGNEFVSAYLQQNQQLDDILTGVNQETVFSAIDFEEDKLSTQTKENQTYYLNYLDTVDKAGKEIYLLEYSTKKELAKDVHDYATKRGWQYYISDSVELDN

SEQ ID NO: 36 - protein, 276 aa, Glycomyces rutgersensis
DSGETATAAPADQPANWIYQLSGYADGKLDALVAAPHEAAVIDLARDGGEGYFSADEITSLENSGKSVYAYFTMGSIETYRPEYDAVAATDMILNQWGDWPDEYFVQYWDQEWWDLVMQPRLDQAAAAGFDGVYLDVPNAYEEIDLALVPGETRESLAQKMVDLVIRAQEYAGDDLQILVQNSPELREYPGYLDAIDGIGIEELFFLNADEPCTEDWCAENLDNTRAIRDAGKLVLAVDYASEPANTAAACEHYAEEGFAGAVAGVDLDAIYEPCP

SEQ ID NO: 37 - protein, 296 aa, Fusarium solani
KPATAARATGLADFKPGVQWEICIHHPIKHDSAADLIPTKAKVWDIDMGHAQEFPNMIPMLKSAGKFVICYFNAGALQDWDDDKSKFPKEVIGHSLSYPYDSEEWYLDIRDSRVLELQTARLDIAAKIGCDAVDPDNVDAWQQDDEDPTGFKLKSSDYTNYLKNLAKYAHSIKTKDGQPLLVGQKNAPEIAEDLVSTLDFAVLESCRGNSDPNEESWPFCEDFQTYIDAGKPVLQIEYPPSVEKTGKVSASDNKYYCTAEDEDKGFSKIIKWASAQLDGWGQYCGEEPFRTPAAKY

SEQ ID NO: 38 - protein, 269 aa, Streptomyces griseofuscus
AAGIKQQVAVPAYFYPGDSGDSGAGNLWAQLSTPAPGAGLAVANPASGPGDSEDGTYANAIRTAHNAGTKVIGYVDSGYLGTKGGAAPDGGTSIDDWVEGAERNVDKWYSYYGGSGLDGIFFDDGLTACGTPSDANAFVDAYKRLQSYVKGKDADAKVVINPGASPEQCYTGAADTLVTFEGTYDDYVNHYGDDRESWEASADPSKIWHLIHTTGSQARMQNAIALSKQRNAGYVYATDDDNSRPSGQDWGNPWDTLPSYWSAEVNTVN

SEQ ID NO: 39 - protein, 313 aa, Microbulbifer hydrolyticus
CNLEDVPNLYPEQGHTDHPQEMRDFVTGIRGYARGLKSGFVVVGHGALPLVSSNERTSGDPDSVYIGNLDALAQDSLFYGHEGIDQPTTDSRRTSLRSYLDMARDTGNTTILITDFAVSEQKIDNAYQLNDDAGYLGFVADHTELDNIPIYPAEPFSVNRRDIFDLDDASNFLVLTNTQLYSTRQDLVDDVADTDYDLIVLDFFFNGEEFTAQQVRQLQRKRNGRTRQVLATVNIGHAESNRYYWENHWVSNPPSWLREEISGSNGDYYVNYWNPAWQDIIYGKNGSYIEKIANAGFDGAYLQGLDAYAHFQN

SEQ ID NO: 40 - protein, 296 aa, Environmental bacterial community
TQVVSNQKDTSKKMQDFVINISKYARKFDADFIIIPQNGEELAFIGANPDKKLNTTFLNAINGFGIEELFYNETFKPNEYRIGLLQKIKDQKTILVSEYVNDTTIVNDAHNKNSNEGFISFIRTKDNYHYSIIPKKINNENSENITSLKDVKNFLYLINNSNFYSKSGFLEAISNTNYDLIFIDLYHNGVLFKKEEIERLKQKKNGGKRLVVCYMNIGAAEKYRNYWKRDWTLGNPSWLKKKYDGYDQEVWVEFWNKDWQKIVYGNDQSYLAKILEAGYDGAYLDNVEAYYFLYND

SEQ ID NO: 41 - protein, 412 aa, Pseudomonas aeruginosa
EIQVLKAPRAVVWKDFLGVNAQFLWFSPERYNKQIDRLQDLGLEWVRLDLHWDRLETAEDQYQLASLDQLVKDLEARQLKSVFYLVGSARFITTAPFYSPFQDQYPPRDPEVFARRMAMLSQRYPSVAAWQVWNEPNLIGFWRPKADPEGYAKLLQASTIALRMVDPEKPVVSAGMAFFSEMPDGRTMFDALGHLGVESLGTIATYHPYTQLPEGNYPWNLDFVSHANQINRALRNAGVPAIWSTEWGWSAYKGPKELQDIIGVEGQADYVLRRLALMSALDYDRIFLFTLSDLDQRASVRDRDYGLLDLDANPKPVYLALQRFLKVTGPKLRPADPPVTEDLPDGSFSIGWTREDGRNVWLFWSARGGNVRLPKLKEATLHDPLSGKVTPLSGSDGLEVPVKSSLQMLVWE

SEQ ID NO: 42 - protein, 412 aa, Pseudomonas fluorescens
ENHVLKGNKVVVWKDFLGVNAQFLWFSPTLYQLQIDRLKALGLQWVRLDLHWDQLEPAEGQYQVATLDQLVANLQTNQLKSVFYLVGSAPFATTAPVGAPYQDQYPPKDPNVFANRMALLSQRYPSVDAWQVWNEPNLLGFWRPAADPAGYANLLTVSAAALHAVNANKPVVAAGMAFFSEMPNGQTMLSALGALGVASLNTVISYHPYTQLPEGNDPANLDFIARTTALNQSLRAAGVHTLWSTEWGWSTYPGPKDAQDLITLQGQADYVVRRVALMSAMDFDKIFLFTLSDLDQRASVRDQSYGLLDIDANPKPVYTALKNFLDVSGPQLTPGDPPAADQLPDGLFSIGWTRADGHKLWYFWSAQGGNAHLPGLTGATLYDPLRGTQTPLSGTGGLTVPVKSNLQILLWD

SEQ ID NO: 43 - protein, 411 aa, Pseudomonas sp.
QTTLKAPRAVEWKNFLGVNAQFQYFDPDNYQKQMTQLDALGLNWIRLTLHWFILEPEQGAFQFSELDAAMAAMKSHGYNTVAYLVGSPPFASSAPAGTPSSDQYPPTDFKLFASRMVSLAQRYPQVSTWQVWNEPNIIWRPKEDPVAYYQMLTTTADALRTQAPGKAIATAGVAYFGQMHSTSGLMLDALLTQGLASQNIIAAYHPYTQFPEGDNAAAQDFLLRGNAMNSDLHGKGVTQVWATEWGWSSYAGPKEMQALIGVDGQADYTLRRLALMSAMDYQRIFLFNLSDLDDRATPRDQFYGLLDLNGEPKPVYNALKNFLTVTGPALQPADAPASNNAPADLYNITWTRNDGAHVWMFWSASGQSLQLPGVTRATLFDPLSGTQTNLSDSTAITVPLKTSLQLLVWTP

SEQ ID NO: 44 - protein, 663 aa, Luteolibacter sp.
ASGVNIHFTDAKPGELEMLKAAGFKHIRMDFGWASTEKQKGVYDFSAYDRLTASLEKHGLKGYYILDYANPLYEKERSVRTEEGRIAYAKWAVAAVTHFKGRGICWEIWNEPNGGFWSPIANVKEYAGMAVMASKAIKQAHPDEYLCGPATSTIDMAFLEGCFKAGLLEWWDAVSVHPYRQGGPESVELEYYALRNLIAKYAPKGKTVSILAGEWGYSSVWMNHDAELQGKMLARQWLVNAANRIPISVWYDWHDDGPDPREAEHHFGTVELKYHEGRDPVYDPKPSYHAAKTFNAVLSGYRFVRRLSLGNTDHQALLFEREGKFILAAWTSVTGERSVRLPSDDGKFTVIGHLGEAMPEVSAKGGALELKVSDAPRYYRFDGANAKLASAPEALLIKVAIVPSTGKELIVKVENLSGKELKAKVMLDRVTELEVDGAPKEIVIPAEMTVTDVVFPLKAIPASNYEAGAKMEVDGVVVSEIVPRLFSPPDDAVLKGARVVGEGDAKIGGSFTLSAAEAPAKFPGGSGAVMKLDYEFVPGWKYAPVYPSDAGRKLEGRPGEEHGRALFGMWIYGDSSHLAPRLRVRDAAGRTWQPSAPEIKWTGWKYVELKLDESTAHWGGEEDKRKRGPKFPLKWEAPFLLDNPQRTAAKGSVWFSMPVVILE

SEQ ID NO: 45 - protein, 414 aa, Pseudomonas sp.
EVTTLKASGPLVWRDFLGVNAQFHFFEPDIYQAQMQQLSDLGLEWVRIAMHWAYLEPKRGQFNLVAFDPMVKAMQQHQLKPVGFLVGSAPFATTAPADSPYQDSFPPKDNALYSESLVRLAKRYDTFEAWQIWNEPNIFPFWRPKEDPQAYAKLLFQSASALRAHVPGKTVVAGGMAYYSNMPSHGGELMLQSLLQMGVAQQKLVMAYHPYTEKPEGASHKQQDYLQHSNFINGALRRHGIEQIWATEWGWSSYKGPREMQAIIGIDGQADYTLRRLALMSAQDFDRIFLFNLSDLDSRAGPRDQGYGLLDLQAKAKPVYNALANLLKVTGPRLEPSDAPRFEQAPKDLYNVTWVREDGSQVWMFWSASGKQLRLPAVTRATLHDPLTGERRELQGAEGIDVPLKSSLQLLVWR

SEQ ID NO: 46 - protein, 413 aa, Pseudomonas frederiksbergensis
VPINLASDRTLEWKDYLGVNAHFLWFTPAQYRKQISAYQKLGLQWVRVDLHWDRLEPKEDDYQLSTLDELDKTLTASGLKSVFYLVGSAPFITRAPVGAPFQDQYPPKDPKVYATRMAMLAQRYPNIDAWQVWNEQNLPNNWRPQVDPAAYGQLLLATHQALDQVAPGKTQVMGGMAYYSQMPTLGKTLMFQALGKLGVQSLGMVAAYHPYSVTPETDEPGKNEVLLRGKQLNDMLHNAGLKNVWATEWGWSSYAGPREMQALIGVDGQADYTLRRLALMSTQDYQRIFLFALSDLDDRASARDQHYGLLDLNGEPKPVYQALARFLDITGPRLKPGKTPVLEGAPDSFYSVAWTRNDGKQLLMFWSAETGTLKLPEIHQASLYDPLTGTQQNLDAADGITPGVKPTLQILVW

SEQ ID NO: 47 - protein, 341 aa, Rhodococcus globerulus
PKPVTTTTTSAPPATCSSVGLGIAGGAPLNWLSQADLDTELSAMKNAGTTWLRFDIDWSAVEPTKGQQNWAATDRVVDRARLQGLSLVGIVTYTPAWARVAGATDTHGYPSDTAAFAKFAQQAAQRYSTRISTWEIWNEPNLTQFFRPKPNVNTYAAILKAASTSIRAVQPGAKILNGGLAPAVDNGSDISPVTYLNALYSAGAKSYFDVFSIHPYSWPALPSDASTSSWNTFYRIRLMRDIMVKNGDTGKKVWATEFGAPTGSGSTAVTPQLQASIISDGFAQAQALGYIERIFIYSMRDRGTNSRDIEQNFGLVTINYTPKPALDAVKKAIGGCSAPKI

SEQ ID NO: 48 - protein, 450 aa, Paenibacillus daejeonensis
APTNTNFGFATGYSILTMSNTDMNAWLDGMAATGAGYIRFDFSWAYIQSGGSTSWNWTQTDRVVDAALAKGFKILPILSHLPGWAGSPSTMNASHFQQFAYQAGLRYIPKGITDWELWNEANIQGFSPANYVNKILIPGANGLRQAASGLNRQVTIVSTGLAPAATNGTHWSMLDYVTGIYANGGKNYFDALGVHPYTWPQNPTVMTNWNWLQKTPELYQVMVNNGDSHKKLWATENGYPTSTTNGVTEQQQAQYIQAAYEIWDSYAFTGGPYFMYSYKDLGTNVQDPEDFFGLVRHNGTLKPAHQTVVNLIAGSTATTYVKIQNRWKDNQFLYDGGTRVQYGNGSGDAYLWALESYNGYTRIRNKATGEYIHIKNGQMQVDSTAIAATDVTSHWTIAGSSATTSAKSIRSRSNGNYLNNEQQLGYVTCDRSTVPHDTAWYSQQWFLVPQ

SEQ ID NO: 49 - protein, 412 aa, Pseudomonas sp.
QGMQLTATRDVVWKDFLGVNAHFLWFPPEHYRQQMQQWKALGLEWTRVDLHWDRHEPRQGQYRLGELDGVIGALADEDLKSVFYLVGSAPHATSAPANSPTPDQYPPKDPVMFAKTMAMLAQRYATVDAWQVWNEPNLPSFWRPHEDAEGYGRLLLPSVQALRQVVPEKPVVMGGMAYFSQMPVKGGLMLEELGKLGVQRLGTVVAYHPYSQEPEYDEPGTNDFILRTQQLNATLRNAQVPGIWATEWGWSSYTGPKELQEIIGEQGQADYVLRRLALMSALDFDRIFLFALADLDSRATARDQHYGLLDLQGQPKPVYTALQRFLTISGPRLQPQQPPRLSVMPDDLYSVAWQREDGRHLWMFWSASGATLQLPELTQAELHDPLTGQQQTLKGANGLSVQAKPGLQMLVW

SEQ ID NO: 50 - protein, 276 aa, Dyella sp.; identical to SEQ ID NO: 36

SEQ ID NO: 51 - protein, 413 aa, Pseudomonas fulva
ANEPFIIGTATHVMDGSPQLAHQFQLASEAGIGSLREDAYWARVELQPGTLQVPASWRAYQKEREARKLGNVVVLDYGNQFYDNNALPRSPMVSTAFANYVDFVTRALAGTVNFYEVWNEWDQAGPGDRAVSDDYASLVKLTRQQIQRNDPKAKVLAGAITSDGLNKGFADRLVQAGLAEQVDGLSLHPYVHCAGKQGKTPESWIKWLSSIDQRLTRLAGKPVPLYLTEMSWPTSSEKTCGVDEPTQAKFLARAYFLAKTRPNIKGMWWYDLVDDGVDPDEREHHFGLLRPGLEPKPAYRVLKAIAPFLAQYQYDSLKSLQTDELYLLNFTKGDEQVLVAWAVGDPRQVKIEANGRQQGPVQMVDTHHPERGRTATGQWQCPKAEEEHCTTVITLDDFPRIISLGDASWLFTR

SEQ ID NO: 52 - protein, 273 aa, Rahnella sp.
VSDSIRKKDSAFLKAKGNGLEPVLILDYGNKFYNDGDYPRNEESINAFVKYATWTATRFKGKVKYYEVWNEWTIGTGMTKYRKNIPSAEIYFNLVKATSEAIKKIDPDAIILAGGFNPLEQRAKFIDVTDTVWFSQLLKLGILNYADGISIHTYSYLNGRRSLRTVEGNLDYLDSFHAASEKIAGKGVPFYITEIGVTNYTGPGGMKEDEAANYIKEYIKSAITRNYIKGVWIYDLIDDGKDKSKRDFNFGLLNNDLSPKQAAPVVSQFLNGK

SEQ ID NO: 53 - protein, 480 aa, Thermobacillus sp.
ADLSQWRLVWSDEFDGPNGSAPDPNKWNLVHAGGGFGNNELQYYTNRRDNSYLENGSLVIKAQKETYNGHAYTSAKLTSQNKGDWKYGRFEIRAKLPYGRSVWPAIWMMPTDSVYGGWPKSGEIDIMENRGDQMNKISGTIHYGNDWPNNTWSGASYNLPGGQSFADDFHTFAIEWEEGIIRWYVDDILYSTKTDWFTPSAPYPAPFDQRFYMQLNVAIGGPNTPFTGFQPPDDSVLPQKMYVDYVRVYERIGSSSSTPIPGKIEAENYSAMNGIQTEQTTDTGGGLNVGWVDAGDWLDYSVNVQTSGTYKVQLRVANALSTGQLQLRSGGTTLATVNVPNTGGWQSWQTIETTVNLTAGQQTLRVYATQRGFNLNWLNFIQDGGSGGGGEHVTADYTAGVSRVSASQAKIYFTPVTPARYVDVHYTVNSGGQLNVRMTNNNGTWETAVNNLKSGDVIRYWFTYEKNGPQYESPEYTYTH

SEQ ID NO: 54 - protein, 262 aa, Paenibacillus sp.
APQQKNGWKLVWNDEFDGKEIDRTKWKHVTGGSGFGNNEDQFYTEDAANSYIEDGKLVIKALKQEHGGKPYTSAKLITEGYADWTYGRFEFRAKMPLGKGMWPAIWMMPTDMEKYGGWPSSGEIDIMEYLGHEPEQVHGTLHMGNPHIYRGGKVSLEDGMFAEAFHDFALEWTPSGMKWYVDDKEFYQTTTWFTRKDEAADNEPFPAPFDRAFFLQLNLAVGGNWPGYPDETTVFPQTFELEYVRVYQPADGNYETANDTAK

SEQ ID NO: 55 - protein, 385 aa, Cohnella sp.
AYNLVWSDEFNGTSIDSNNWSFEVGTGSGGWGNNELEYYTSRSENARIENGNLVIEARKESYGGMNYTSARLKTQGKKSFQYGRIEARIKMPNGQGLWPAFWTLGSDIGTVGWPKSGEIDIMEHVNNDNNTNGYIHWDANGQADYGGPSGYVDVTQYHVYSIEWTPSAIKWFIDGTQFWEANIANNINSTEEFHKPHFILLNMAVGGNWPGAPNAGTAFPAKMYVDYVRVYQDNGTPQPSNGIVSGGTYKLINVNSGKALDVQSAGTTPGTNVQIWTDNGTGAQKWTIYQNADGSYKLVNVNSALALDVASSGTADGTNVQAWTDNGTGAQKWNIIANGDGSYKLINTNSGKALDVSGSGTADGTNVQIWNDNGTGAQKWNLIKL

SEQ ID NO: 56 - protein, 382 aa, Paenibacillus elgii
APNWNLVWSDEFNGNALNSANWSAEIGTGQNGWGNNELQYYTNRPENVRVADGNLVITARKESYGGMNYTSARIKTQNLKSFTYGKIEARIKLPSGQGLWPAFWMLGSNINAVGWPGCGEIDIMERVNNNPHVNGTVHWDAGGHADYGRVSGNLDFSQYHVYSIEWDSKYIRWFVDGQEYNAFYIENGTGNTEEFQRPFFLLLNLAVGGNWPGSPDPSTPFPAQMLVDYVRVYQASPGIVNGGIYTIASKASGKVMDVVDVSTQSGAKIQQWTNYVANNQKFKVESAGDGYYKLTAVHSGKVLDVPNSSTSSGVQLQQWDDNGSAAQRWSIVDAGGGYYKIVSKTNGLVVDVSGSSTADGATVQQWSDNGTDAQKWSFVKVN

SEQ ID NO: 57 - protein, 260 aa, Bacillus species A
TETEEGISIEQEGWNLVWNDEFDGDSLDQSKWRYDIGNGQPNLPGWGNEELQYYNDDPKNVRVENGELIIEAHQEPISDEFGSYEYTSGKVLTEGLFSQTYGRFEARMRLPAGQGFWPAFWMMPENDQYGGWAASGEIDIMENAGGTPYKVGGAIHYGGPWPENQFQAGDYFFPDGTDATGYHEYAVEWEPGEIRWYVDGNLYQTINDWYSTGGAYPAPFDQDFHLILNLAVGGWYGGNPDGSTPFPSTMAVDYVRVYER

SEQ ID NO: 58 - protein, 256 aa, Bacillus species B
ATAPEPQNDWNLVWSDEFDGNSLDSSKWRYDIGNGQPNLPGWGNEELQYYSDDPKNVRVENGELVIEAHQETVSDPYGTYPYTSGKVLTDGKFSQTYGRFEARMRLPAGQGFWPAFWMMPENDRYGGWAASGEIDIMENAGATPYKTGGAIHYGGPWPENQFQAGDYYFPDWTNATDYHEYAVEWEPGEIRWYVDGNLYQTINDWYSVGGSYPAPFDQDFHLILNLAVGGWYGGNPDATTPFPSTMAVDYVRVYQR

SEQ ID NO: 59 - protein, 763 aa, Paenibacillus sp.
MKRSYATERRYLQKGLSLFFAVVMLASVGLWPASKVEAADFTVTSMDYFSAADGPVISKSGVGQASYGFVMPIFNGGAATWNDVAQDVGVKVKVGGSWVDIDSVSSFIYNQNWGHWSDGGFTGYWFTLSATTEIQLYSKANGVTLDYRLVFQNINKTTITAMTPTQGPQITASFTGGAGFTYPTFNNDPAVTYAAVADDLKVFVKPVNSSTWIDIDNNAASGWIYDHNFGQFTDGGGGYWFNVTESIHVKLESKTSGVNVVYTITFNEAVRNSYVITPYEGTTFTADANGSIGIPLPKIDGGAPIGKELDNFVYQININGQWVELGNSGQSGFTYAANGYNNMSDANQWGYWADYIYGLWFQPIQEDMQIRIGYPLNGQKGGSVGSNYVNYTLIGNPDAPRPDVSDQEDIAIGTPSDPAIQGMNLIWQDEFNGTTLDTSKWNYEQGYYLNDDPNTWGWGNAELQHYTDSAQNVFVQDGKLNIRALNDPKSFPQDPSRYAQYSSGKINTKNHFTLKYGRVDFRAKLPTGNGVWPALWMLPQDSPYGTWAASGEIDVMEARGRLPGSTSGAVHFGGTWPANQHISGEYHFPEGQNINNDYHVYSVVWEEDNIKWYVDGKFFFKVTNEQWYSLAAPNNPNAPFDQPFYLIMNLALGGNFDGGISPNPSDIPVTMQVDYVRVYKENGSGNPGNVPVTGVTLNPTSAQVEVGQSLQLNAGIAPSNATNKQVTWSVSGASVASVSQEGVVTGLAPGTATVTATSVDGQK

SEQ ID NO: 60 - protein, 876 aa, Paenibacillus sp.
MNRHVLLHPYLHRKALPLLLALTLLTGIALFPASTAQAATTVTSMTYFSANDGPVISKSGVGQASYGFVMPIFNGGAATWNDVADDVGVRVKVGGSWVDIDSVGGYVYNQNWGHWNDSGTYGYWFTLSATTELQLYSKANSSVTLNYTLVFQNVNETTITSMTPTQGPQLTAGYTGGAGFTYPVFNNDPSIPYAAVAGDLKVYVKPVASSTWIDIDNNAASGWIYDSNFGQFTEGGGGYWFTVTESINVKLESRTSSANVVYTINFPQPTRSSYTLSAYDGTTYSADASGAIGIPLPRIDGTPAIGSELGNFVYQIYRNGQWVEMSNSAQSSFVYSANGYNNMSDANQWGYWADYIYGLWFRPIQEDMQIRIGYPLNGQSGGSVGSNFVTYTLIGNPNAPRPDVSDQGDVEIGTPTDPAIAGWNLYWQDEFAGSALDLNKWNYETGYYIGNDPNLWGWGNAEMQHYTTSTQNVFVADGKLNIRALHDYQSFPQDPNRYATYSSGKINTKDNMSLQYGRVDIRAKLPTGDGVWPALWMLPEDSVYGAWAASGEIDIMEAKGRLPGTTSGAIHYGGQWPVNRYLAGECYLPQGTTFADDFNVYTMIWEEDNMKWYVNGEFFFKVTREQWYSVAAPNNPDAPFDQPFYLIMNLAVGGHFDGGRTPDPSDIPATMQIDYVRVYKEGAGGGPGNPGGNVAVTGVSVTPATAQVQVGQTVSLSANVAPANATNKQVTWSVANGSIASVSASGVVSGLAAGTTTVTATTADGNRTASATITVVPPPTTTVIIGDSVRGIRKTGDNLLFYVNGATYADLHYKVNGGGQPNVAMTHTGGGNYTYPVHGLQQGDTVEYFFTYNPGNGALDTPWQTYVHGVTQGVVE

SEQ ID NO: 61 - protein, 482 aa, Zobellia galactanivorans
MKKIITYLLMVLCFGMTPILSAQDYNLVWQDEFDDGIGPDWVFETGMGYNGWGNNELQYYRRENAAVENGNLVITAKHENFGGAQYTSARMKTQGRKSFKYGKIEARIALPSGQGLWPAFWMLGNNITSVSWPACGEIDIMERINNALQTHGTIHWSDQNGDHASYGDDVGVSDPGQYHIYSVEWDANSIKWFVDGQQFNEVDISNGVNGTGEFQNEFFILLNMAVGGDWPGFDVDQSKLPAQMLVDYVRVYQKGDDNDSANTLKIEAESYLYSNDVQKEPCSEGGENVGYINNGSWMSYPGINFPSSGNYLIEYRVASAVDGGRFSSDLEAGETVLGELSVPNTGGWQNWTTVSQTVNVSAGTYQFGLYSISGGWNINWIRITKQGTASAATALNSSLIASDNGISQEIRVYPNPFTEYVSVNFDGEAANLTLQDMLGTVIFSKSGVSADESVDLSGLKSGVYFLTIEQDGKSTVRQLIKE

SEQ ID NO: 62 - protein, 449 aa, Paenibacillus sp.
MKQKGMRYLLVLSLLLTCWSVFGTRAEAADYTQGVELSGSTATVWFKSAVNTSWVDVHYRVNGGEQQNVRMSYHAGKSRYEQAISGIAAGHVITYSFTYNNGIPAYDTGVFSYTAGSTPPPSSSGSIYDILPSTIPMPPNGAVSVKIMNGTHGAYTDQQIYWGVLGINPVNNQWSYLDLNGNLIPISSALNDAPGHLTKNGINYANIYHKVNDASWVTLPQITSGRMFLSVGTPLYLKTFNDGFAGPDLNNPTDPNRDIYFDFVEFTIDAAGYHGNTTRVDGFGFPLQHRLVNKSGSFDQTVGELESETRNGIFAKFQAEVPAAFKSLATIQAPYRIVAPIHGSFAQGGANANYFGGYAPYSTQDIFRCDGALTDAATCAAIQRHVYTANDWNNVSNYYQAAPANYYAKFWHDHSINRLAYGFPYDDVNGQAAYLEVGDPKGLIIRIGW

SEQ ID NO: 63 - protein, 641 aa, Thermotoga petrophila [sequence omitted]

SEQ ID NO: 64 - protein, 286 aa, Rhodothermus marinus
MCTMPLMKLKKMMRRTAFLLSVLIGCSMLGSDRSDKAPHWELVWSDEFDYSGLPDPEKWDYDVGGHGWGNQELQYYTRARIENARVGGGVLIIEARHEPYEGREYTSARLVTRGKASWTYGRFEIRARLPSGRGTWPAIWMLPDRQTYGSAYWPDNGEIDIMEHVGFNPDVVHGTVHTKAYNHLLGTQRGGSIRVPTARTDFHVYAIEWTPEEIRWFVDDSLYYRFPNERLTDPEADWRHWPFDQPFHLIMNIAVGGAWGGQQGVDPEAFPAQLVVDYVRVYRWVE

SEQ ID NO: 65 - protein, 291 aa, Trichoderma sp.
MWSPKVAAAVLAFVGATNAWQPPTYSGFNLVWTDTFAGGGTSPNQNNWNIITGNLNVNAEQETYSSSTANVQLSGGSTLQLVPWRDSSKGTSTFGGWTSGRLESKYTFTPAAGKVTRLEAAIRFGSNAQANKQGIWPAFWMLGDSLRQPGGSWPNCGEIDIMETVDGQATGHGTLHCDVYPGGICNEGNGIGGPVNIANVNDWHAWRVEIDRTPSSWQSETLTWSLDGTIYFQITGSRIGNQGVWNNIAHSPLFFILNVAVGGNWPGNPNSATLDGYGSMMEVGYVAQYST

SEQ ID NO: 66 - protein, 324 aa, Terribacillus saccharophilus [sequence omitted]

SEQ ID NO: 67 - protein, 672 aa, Escherichia coli
MLRNGNKYLLMLVSIIMLTACISQSRTSFIPPQDRESLLAEQPWPHNGFVAISWHNVEDEAADQRFMSVRTSALREQFAWLRENGYQPVSIAQIREAHRGGKPLPEKAVVLTFDDGYQSFYTRVFPILQAFQWPAVWAPVGSWVDTPADKQVKFGDELVDREYFATWQQVREVARSRLVELASHTWNSHYGIQANATGSLLPVYVNRAYFTDHARYETAAEYRERIRLDAVKMTEYLRTKVEVNPHVFVWPYGEANGIAIEELKKLGYDMFFTLESGLANASQLDSIPRVLIANNPSLKEFAQQIITVQEKSPQRIMHIDLDYVYDENLQQMDRNIDVLIQRVKDMQISTVYLQAFADPDGDGLVKEVWFPNRLLPMKADIFSRVAWQLRTRSGVNIYAWMPVLSWDLDPTLTRVKYLPTGEKKAQIHPEQYHRLSPFDDRVRAQVGMLYEDLAGHAAFDGILFHDDALLSDYEDASAPAITAYQQAGFSGSLSEIRQNPEQFKQWARFKSRALTDFTLELSARVKAIRGPHIKTARNIFALPVIQPESEAWFAQNYADFLKSYDWTAIMAMPYLEGVAEKSADQWLIQLTNQIKNIPQAKDKSILELQAQNWQKNGQHQAISSQQLAHWMSLLQLNGVKNYGYYPDNFLHNQPEIDLIRPEFSTAWYPKND